European Patent Application EP 4 711 446 A1, published March 18, 2026. Title: CELL CULTURE PRODUCT AND USE THEREOF. Applicant: GUANGXIU-GAOXIN LIFE SCIENCES CO., LTD. HUNAN. The sequence listing filed with the application follows.

SEQUENCE LISTING (24 sequences)

SEQ ID NO: 1 - DNA, 20 bp, synthetic construct
  source 1..20: mol_type = other DNA
agcgaaccagtatcgagaac

SEQ ID NO: 2 - DNA, 20 bp, synthetic construct
  source 1..20: mol_type = other DNA
ttacagaaccacactcggac

SEQ ID NO: 3 - DNA, 21 bp, synthetic construct
  source 1..21: mol_type = other DNA
ggtctcgtatttgctgcatcg

SEQ ID NO: 4 - DNA, 20 bp, synthetic construct
  source 1..20: mol_type = other DNA
acactcggtgaaatcagggt

SEQ ID NO: 5 - DNA, 20 bp, synthetic construct
  source 1..20: mol_type = other DNA
agctacagcatgatgcagga

SEQ ID NO: 6 - DNA, 20 bp, synthetic construct
  source 1..20: mol_type = other DNA
ggtcatggagttgtactgca

SEQ ID NO: 7 - DNA, 20 bp, synthetic construct
  source 1..20: mol_type = other DNA
ggaccgcacggaatttgaac

SEQ ID NO: 8 - DNA, 20 bp, synthetic construct
  source 1..20: mol_type = other DNA
ggacaccaccgaggaaatgg

SEQ ID NO: 9 - DNA, 22 bp, synthetic construct
  source 1..22: mol_type = other DNA
ggaacaccactacgccttcaac

SEQ ID NO: 10 - DNA, 22 bp, synthetic construct
  source 1..22: mol_type = other DNA
tcatgttgctcacggaggagta

SEQ ID NO: 11 - DNA, 21 bp, synthetic construct
  source 1..21: mol_type = other DNA
ccatgtacatgagcactgttg

SEQ ID NO: 12 - DNA, 21 bp, synthetic construct
  source 1..21: mol_type = other DNA
ctccaataactcctggtatcc

SEQ ID NO: 13 - DNA, 21 bp, synthetic construct
  source 1..21: mol_type = other DNA
catggccaagattgacaacct

SEQ ID NO: 14 - DNA, 22 bp, synthetic construct
  source 1..22: mol_type = other DNA
ttcccatatgttcctgcatcag

SEQ ID NO: 15 - DNA, 21 bp, synthetic construct
  source 1..21: mol_type = other DNA
catggccaagattgacaacct

SEQ ID NO: 16 - DNA, 22 bp, synthetic construct
  source 1..22: mol_type = other DNA
ttcccatatgttcctgcatcag

SEQ ID NO: 17 - DNA, 22 bp, synthetic construct
  source 1..22: mol_type = other DNA
gatgagatgcctgctgacttgc

SEQ ID NO: 18 - DNA, 23 bp, synthetic construct
  source 1..23: mol_type = other DNA
cacgacagagtaatcaggatgcc

SEQ ID NO: 19 - DNA, 22 bp, synthetic construct
  source 1..22: mol_type = other DNA
gatgagatgcctgctgacttgc

SEQ ID NO: 20 - DNA, 23 bp, synthetic construct
  source 1..23: mol_type = other DNA
cacgacagagtaatcaggatgcc

SEQ ID NO: 21 - DNA, 23 bp, synthetic construct
  source 1..23: mol_type = other DNA
cgtgcatgtgttcagaaaggctg

SEQ ID NO: 22 - DNA, 22 bp, synthetic construct
  source 1..22: mol_type = other DNA
ctcctcagttgtgagcccatgc

SEQ ID NO: 23 - DNA, 22 bp, synthetic construct
  source 1..22: mol_type = other DNA
agtgagcagcttccgagtcaag

SEQ ID NO: 24 - DNA, 22 bp, synthetic construct
  source 1..22: mol_type = other DNA
gagaactccgcgacgatgttgt